European Patent Application EP 4 737 573 A1, published May 6, 2026. Title: グラム陰性菌の外膜透過性ポリペプチド、該ポリペプチドを含む抗菌性タンパク質、抗菌剤又は消毒剤、医薬組成物並びに抗菌剤組成物又は消毒剤組成物. Applicant: 国立大学法人岡山大学. The sequence listing filed with the application follows.

SEQUENCE LISTING (10 sequences)

SEQ ID NO: 1 - protein, 133 aa, synthetic construct
NSGTPKNVSRGTSSTKTTPKYKVKNGDNLTKIAKKHNTTVATLLKLNPGIKDPNMIRVGQTLNVTGSGGKTHKVKSGDTLSKIAVDNKTTVSKLMNLNPEITNPNHIKVGQTIRLSRKLRRLKRKIAHKVKKY

SEQ ID NO: 2 - DNA, 399 bp, synthetic construct
  source 1..399: mol_type = other DNA
aattctggcacgcctaagaacgtatcgcgcggcacgtcatccacgaagacgacgcctaagtacaaggtaaagaacggcgataatctcaccaaaattgccaagaaacacaatacgacagtggctactttattaaaactcaatccaggcattaaagatccgaacatgattcgtgtcggtcaaacattaaatgtgacagggagcggcggtaagacacacaaagtaaagagtggtgataccttgagcaagattgccgtggataataagactacagttagtaagttgatgaatttgaatcctgagatcacaaatcctaatcatatcaaagtagggcagaccattcgcttaagccggaagctccgtcggcttaaacgtaagatcgctcacaaggtaaaaaaatat

SEQ ID NO: 3 - protein, 116 aa, Bacillus amyloliquefaciens phage Morita2001
NSGTPKNVSRGTSSTKTTPKYKVKNGDNLTKIAKKHNTTVATLLKLNPGIKDPNMIRVGQTLNVTGSGGKTHKVKSGDTLSKIAVDNKTTVSKLMNLNPEITNPNHIKVGQTIRLS

SEQ ID NO: 4 - protein, 17 aa, synthetic construct
RKLRRLKRKIAHKVKKY

SEQ ID NO: 5 - DNA, 432 bp, Pseudomonas aeruginosa phage PAJU2
  source 1..432: mol_type = genomic DNA
atgcgtacatcccaacgaggcatcgacctcatcaaatccttcgagggcctgcgcctgtccgcttaccaggactcggtgggtgtctggaccataggttacggcaccactcggggcgtcacccgctacatgacgatcaccgtcgagcaggccgagcggatgctgtcgaacgacattcagcgcttcgagccagagctagacaggctggcgaaggtgccactgaaccagaaccagtgggatgccctgatgagcttcgtgtacaacctgggcgcggccaatctggcgtcgtccacgctgctcaagctgctgaacaagggtgactaccagggagcagcggaccagttcccgcgctgggtgaatgcgggcggtaagcgcttggatggtctggttaagcgtcgagcagccgagcgtgcgctgttcctggagccactatcg

SEQ ID NO: 6 - DNA, 348 bp, Bacillus amyloliquefaciens phage Morita2001
  source 1..348: mol_type = genomic DNA
aattctggcacgcctaagaacgtatcgcgcggcacgtcatccacgaagacgacgcctaagtacaaggtaaagaacggcgataatctcaccaaaattgccaagaaacacaatacgacagtggctactttattaaaactcaatccaggcattaaagatccgaacatgattcgtgtcggtcaaacattaaatgtgacagggagcggcggtaagacacacaaagtaaagagtggtgataccttgagcaagattgccgtggataataagactacagttagtaagttgatgaatttgaatcctgagatcacaaatcctaatcatatcaaagtagggcagaccattcgcttaagc

SEQ ID NO: 7 - DNA, 51 bp, synthetic construct
  source 1..51: mol_type = other DNA
cggaagctccgtcggcttaaacgtaagatcgctcacaaggtaaaaaaatat

SEQ ID NO: 8 - protein, 297 aa, synthetic construct
HMELGTLEMRTSQRGIDLIKSFEGLRLSAYQDSVGVWTIGYGTTRGVTRYMTITVEQAERMLSNDIQRFEPELDRLAKVPLNQNQWDALMSFVYNLGAANLASSTLLKLLNKGDYQGAADQFPRWVNAGGKRLDGLVKRRAAERALFLEPLSKLVDNSGTPKNVSRGTSSTKTTPKYKVKNGDNLTKIAKKHNTTVATLLKLNPGIKDPNMIRVGQTLNVTGSGGKTHKVKSGDTLSKIAVDNKTTVSKLMNLNPEITNPNHIKVGQTIRLSRKLRRLKRKIAHKVKKYSRHHHHHH

SEQ ID NO: 9 - protein, 285 aa, synthetic construct
HMMRTSQRGIDLIKSFEGLRLSAYQDSVGVWTIGYGTTRGVTRYMTITVEQAERMLSNDIQRFEPELDRLAKVPLNQNQWDALMSFVYNLGAANLASSTLLKLLNKGDYQGAADQFPRWVNAGGKRLDGLVKRRAAERALFLEPLSNSGTPKNVSRGTSSTKTTPKYKVKNGDNLTKIAKKHNTTVATLLKLNPGIKDPNMIRVGQTLNVTGSGGKTHKVKSGDTLSKIAVDNKTTVSKLMNLNPEITNPNHIKVGQTIRLSRKLRRLKRKIAHKVKKYHHHHHH

SEQ ID NO: 10 - DNA, 855 bp, synthetic construct
  source 1..855: mol_type = other DNA
atgatgcgtacatcccaacgaggcatcgacctcatcaaatccttcgagggcctgcgcctgtccgcttaccaggactcggtgggtgtctggaccataggttacggcaccactcggggcgtcacccgctacatgacgatcaccgtcgagcaggccgagcggatgctgtcgaacgacattcagcgcttcgagccagagctagacaggctggcgaaggtgccactgaaccagaaccagtgggatgccctgatgagcttcgtgtacaacctgggcgcggccaatctggcgtcgtccacgctgctcaagctgctgaacaagggtgactaccagggagcagcggaccagttcccgcgctgggtgaatgcgggcggtaagcgcttggatggtctggttaagcgtcgagcagccgagcgtgcgctgttcctggagccactatcgaattctggcacgcctaagaacgtatcgcgcggcacgtcatccacgaagacgacgcctaagtacaaggtaaagaacggcgataatctcaccaaaattgccaagaaacacaatacgacagtggctactttattaaaactcaatccaggcattaaagatccgaacatgattcgtgtcggtcaaacattaaatgtgacagggagcggcggtaagacacacaaagtaaagagtggtgataccttgagcaagattgccgtggataataagactacagttagtaagttgatgaatttgaatcctgagatcacaaatcctaatcatatcaaagtagggcagaccattcgcttaagccggaagctccgtcggcttaaacgtaagatcgctcacaaggtaaaaaaatatcatcatcatcatcatcattag